European Patent Application EP 4 745 152 A2, published May 20, 2026. Title: PEPTIDES BINDING TO BFL-1. Applicant: Dana-Farber Cancer Institute, Inc. Application EP. The sequence listing filed with the application follows.

SEQUENCE LISTING (210 sequences)

SEQ ID NO: 1 - protein, 25 aa, synthetic construct
  REGION 1..25: note = Description of Artificial Sequence: Syntheticpeptide
AELEVESATQLRRFGDKLNFRQKLL

SEQ ID NO: 2 - protein, 26 aa, synthetic construct
  REGION 1..26: note = Description of Artificial Sequence: Syntheticpeptide
DMPREIWIAQELRRIGDEFNAYYARR

SEQ ID NO: 3 - protein, 27 aa, synthetic construct
  REGION 1..27: note = Description of Artificial Sequence: Syntheticpeptide
QDASTKKLSESLKRIGDELDSNMELQR

SEQ ID NO: 4 - protein, 34 aa, synthetic construct
  REGION 1..34: note = Description of Artificial Sequence: Syntheticpolypeptide
SSTMGQVGRQLAIIGDDINRRYDSEFQTMLQHLQ

SEQ ID NO: 5 - protein, 25 aa, synthetic construct
  REGION 1..25: note = Description of Artificial Sequence: Syntheticpeptide
PGGRLAEVSTVLLRLGDELEQIRPS

SEQ ID NO: 6 - protein, 29 aa, synthetic construct
  REGION 1..29: note = Description of Artificial Sequence: Syntheticpeptide
SESQEDIIRNIARHLAQVGDSMDRSIPPG

SEQ ID NO: 7 - protein, 33 aa, synthetic construct
  REGION 1..33: note = Description of Artificial Sequence: Syntheticpolypeptide
EEEQWAREIGAQLRRMADDLNAQYERRRQEEQQ

SEQ ID NO: 8 - protein, 30 aa, synthetic construct
  REGION 1..30: note = Description of Artificial Sequence: Syntheticpolypeptide
KKFEPKSGWMTFLEVTGKICEMLSLLKQYC

SEQ ID NO: 9 - protein, 25 aa, synthetic construct
  REGION 1..25: note = Description of Artificial Sequence: Syntheticpeptide
  MOD_RES 13: note = Any non-natural amino acid
  MOD_RES 17: note = Any non-natural amino acid
AELEVECATQLRXFGDXLNFRQKLL

SEQ ID NO: 10 - protein, 25 aa, synthetic construct
  REGION 1..25: note = Description of Artificial Sequence: Syntheticpeptide
  MOD_RES 13: note = Any non-natural amino acid
  MOD_RES 17: note = Any non-natural amino acid
AELEVECATQLRXFGDXLNFRQKDL

SEQ ID NO: 11 - protein, 25 aa, synthetic construct
  REGION 1..25: note = Description of Artificial Sequence: Syntheticpeptide
  MOD_RES 13: note = Any non-natural amino acid
  MOD_RES 17: note = Any non-natural amino acid
AELEVELATQLRXFGDXLNFRQKLL

SEQ ID NO: 12 - protein, 25 aa, synthetic construct
  REGION 1..25: note = Description of Artificial Sequence: Syntheticpeptide
  MOD_RES 13: note = Any non-natural amino acid
  MOD_RES 17: note = Any non-natural amino acid
AELEVECLTQLRXFGDXLNFRQKLL

SEQ ID NO: 13 - protein, 25 aa, synthetic construct
  REGION 1..25: note = Description of Artificial Sequence: Syntheticpeptide
  MOD_RES 13: note = Any non-natural amino acid
  MOD_RES 17: note = Any non-natural amino acid
AELEVESATQLRXFGDXLNFRQKLL

SEQ ID NO: 14 - protein, 23 aa, synthetic construct
  REGION 1..23: note = Description of Artificial Sequence: Syntheticpeptide
  MOD_RES 11: note = Any non-natural amino acid
  MOD_RES 15: note = Any non-natural amino acid
LEVECATQLRXFGDXLNFRQKLL

SEQ ID NO: 15 - protein, 22 aa, synthetic construct
  REGION 1..22: note = Description of Artificial Sequence: Syntheticpeptide
  MOD_RES 13: note = Any non-natural amino acid
  MOD_RES 17: note = Any non-natural amino acid
AELEVECATQLRXFGDXLNFRQ

SEQ ID NO: 16 - protein, 25 aa, synthetic construct
  REGION 1..25: note = Description of Artificial Sequence: Syntheticpeptide
  MOD_RES 13: note = Any non-natural amino acid
  MOD_RES 17: note = Any non-natural amino acid
AELEVECATQLRXYGDXLNFRQKLL

SEQ ID NO: 17 - protein, 25 aa, synthetic construct
  REGION 1..25: note = Description of Artificial Sequence: Syntheticpeptide
  MOD_RES 13: note = Any non-natural amino acid
  MOD_RES 17: note = Any non-natural amino acid
AELEVECATQLRXIGDXLNFRQKLL

SEQ ID NO: 18 - protein, 20 aa, synthetic construct
  REGION 1..20: note = Description of Artificial Sequence: Syntheticpeptide
  MOD_RES 9: note = Any non-natural amino acid
  MOD_RES 13: note = Any non-natural amino acid
VECATQLRXFGDXLNFRQKL

SEQ ID NO: 19 - protein, 20 aa, synthetic construct
  REGION 1..20: note = Description of Artificial Sequence: Syntheticpeptide
  MOD_RES 9: note = Any non-natural amino acid
  MOD_RES 13: note = Any non-natural amino acid
VECATQLRXFGFXLNFRQKL

SEQ ID NO: 20 - protein, 25 aa, synthetic construct
  REGION 1..25: note = Description of Artificial Sequence: Syntheticpeptide
  MOD_RES 6: note = Any non-natural amino acid
  MOD_RES 10: note = Any non-natural amino acid
AELEVXCATXLRRFGDKLNFRQKLL

SEQ ID NO: 21 - protein, 25 aa, synthetic construct
  REGION 1..25: note = Description of Artificial Sequence: Syntheticpeptide
  MOD_RES 19: note = Any non-natural amino acid
  MOD_RES 23: note = Any non-natural amino acid
AELEVECATQLRRFGDKLXFRQXLL

SEQ ID NO: 22 - protein, 24 aa, synthetic construct
  REGION 1..24: note = Description of Artificial Sequence: Syntheticpeptide
  MOD_RES 1: note = Non-natural electrophile containing amino acid or not present
  MOD_RES 11: note = Any non-natural amino acid
  MOD_RES 15: note = Any non-natural amino acid
XEVESATQLRXFGDXLNFRQKLLK

SEQ ID NO: 23 - protein, 20 aa, synthetic construct
  REGION 1..20: note = Description of Artificial Sequence: Syntheticpeptide
  MOD_RES 1: note = Non-natural electrophile containing amino acid or not present
  MOD_RES 7: note = Any non-natural amino acid
  MOD_RES 11: note = Any non-natural amino acid
XATQLRXFGDXLNFRQKLLK

SEQ ID NO: 24 - protein, 23 aa, synthetic construct
  REGION 1..23: note = Description of Artificial Sequence: Syntheticpeptide
  MOD_RES 1: note = Non-natural electrophile containing amino acid or not present
  MOD_RES 11: note = Any non-natural amino acid
  MOD_RES 15: note = Any non-natural amino acid
XEVESATQLRXFGDXLNFRQKLL

SEQ ID NO: 25 - protein, 19 aa, synthetic construct
  REGION 1..19: note = Description of Artificial Sequence: Syntheticpeptide
  MOD_RES 1: note = Non-natural electrophile containing amino acid or not present
  MOD_RES 7: note = Any non-natural amino acid
  MOD_RES 11: note = Any non-natural amino acid
XATQLRXFGDXLNFRQKLL

SEQ ID NO: 26 - protein, 17 aa, synthetic construct
  REGION 1..17: note = Description of Artificial Sequence: Syntheticpeptide
  MOD_RES 1: note = Non-natural electrophile containing amino acid or not present
  MOD_RES 8: note = Any non-natural amino acid
  MOD_RES 12: note = Any non-natural amino acid
XLSESLKXIGDXLDSNK

SEQ ID NO: 27 - protein, 19 aa, synthetic construct
  REGION 1..19: note = Description of Artificial Sequence: Syntheticpeptide
  MOD_RES 1: note = Non-natural electrophile containing amino acid or not present
  MOD_RES 7: note = Any non-natural amino acid
  MOD_RES 11: note = Any non-natural amino acid
XAQELRXIGDXFNAYYARK

SEQ ID NO: 28 - protein, 20 aa, synthetic construct
  REGION 1..20: note = Description of Artificial Sequence: Syntheticpeptide
  MOD_RES 1: note = Non-natural electrophile containing amino acid or not present
  MOD_RES 8: note = Any non-natural amino acid
  MOD_RES 12: note = Any non-natural amino acid
XIAQELRXIGDXFNAYYARK

SEQ ID NO: 29 - protein, 19 aa, synthetic construct
  REGION 1..19: note = Description of Artificial Sequence: Syntheticpeptide
  MOD_RES 1: note = Non-natural electrophile containing amino acid or not present
  MOD_RES 7: note = Any non-natural amino acid
  MOD_RES 11: note = Any non-natural amino acid
XAQELRXIGDXFNAYYARR

SEQ ID NO: 30 - protein, 20 aa, synthetic construct
  REGION 1..20: note = Description of Artificial Sequence: Syntheticpeptide
  MOD_RES 1: note = Non-natural electrophile containing amino acid or not present
  MOD_RES 8: note = Any non-natural amino acid
  MOD_RES 12: note = Any non-natural amino acid
XIAQELRXIGDXFNAYYARR

SEQ ID NO: 31 - protein, 16 aa, synthetic construct
  REGION 1..16: note = Description of Artificial Sequence: Syntheticpeptide
  MOD_RES 1: note = Non-natural electrophile containing amino acid or not present
  MOD_RES 4: note = Any non-natural amino acid
  MOD_RES 8: note = Any non-natural amino acid
XVGXQLAXIGDDINRR

SEQ ID NO: 32 - protein, 15 aa, synthetic construct
  REGION 1..15: note = Description of Artificial Sequence: Syntheticpeptide
  MOD_RES 1: note = Non-natural electrophile containing amino acid or not present
  MOD_RES 3: note = Any non-natural amino acid
  MOD_RES 7: note = Any non-natural amino acid
  MOD_RES 15: note = May or may not be present
XGXQLAXIGDDINRR

SEQ ID NO: 33 - protein, 16 aa, synthetic construct
  REGION 1..16: note = Description of Artificial Sequence: Syntheticpeptide
  MOD_RES 1: note = Non-natural electrophile containing amino acid or not present
XEVSTVLLRLGDELEQ

SEQ ID NO: 34 - protein, 15 aa, synthetic construct
  REGION 1..15: note = Description of Artificial Sequence: Syntheticpeptide
  MOD_RES 1: note = Non-natural electrophile containing amino acid or not present
XVSTVLLRLGDELEQ

SEQ ID NO: 35 - protein, 14 aa, synthetic construct
  REGION 1..14: note = Description of Artificial Sequence: Syntheticpeptide
  MOD_RES 1: note = Non-natural electrophile containing amino acid or not present
XSTVLLRLGDELEQ

SEQ ID NO: 36 - protein, 13 aa, synthetic construct
  REGION 1..13: note = Description of Artificial Sequence: Syntheticpeptide
  MOD_RES 1: note = Non-natural electrophile containing amino acid or not present
XTVLLRLGDELEQ

SEQ ID NO: 37 - protein, 16 aa, synthetic construct
  REGION 1..16: note = Description of Artificial Sequence: Syntheticpeptide
GQVGRQLAIIGDDINR

SEQ ID NO: 38 - protein, 21 aa, synthetic construct
  REGION 1..21: note = Description of Artificial Sequence: Syntheticpeptide
IWIAQELRRIGDEFNAYYARR

SEQ ID NO: 39 - protein, 16 aa, synthetic construct
  REGION 1..16: note = Description of Artificial Sequence: Syntheticpeptide
KLSECLKRIGDELDSN

SEQ ID NO: 40 - protein, 16 aa, synthetic construct
  REGION 1..16: note = Description of Artificial Sequence: Syntheticpeptide
LAECTVLLRLGDELEQ

SEQ ID NO: 41 - protein, 22 aa, synthetic construct
  REGION 1..22: note = Description of Artificial Sequence: Syntheticpeptide
  MOD_RES 1: note = Non-natural electrophile containing amino acid or not present
XDIIRNIARHLAQVGDSMDRSI

SEQ ID NO: 42 - protein, 22 aa, synthetic construct
  REGION 1..22: note = Description of Artificial Sequence: Syntheticpeptide
  MOD_RES 3: note = Non-natural electrophile containing amino acid or not present
EDXIRNIARHLAQVGDSMDRSI

SEQ ID NO: 43 - protein, 22 aa, synthetic construct
  REGION 1..22: note = Description of Artificial Sequence: Syntheticpeptide
  MOD_RES 6: note = Non-natural electrophile containing amino acid or not present
EDIIRXIARHLAQVGDSMDRSI

SEQ ID NO: 44 - protein, 22 aa, synthetic construct
  REGION 1..22: note = Description of Artificial Sequence: Syntheticpeptide
  MOD_RES 7: note = Non-natural electrophile containing amino acid or not present
EDIIRNXARHLAQVGDSMDRSI

SEQ ID NO: 45 - protein, 19 aa, synthetic construct
  REGION 1..19: note = Description of Artificial Sequence: Syntheticpeptide
  MOD_RES 1: note = Non-natural electrophile containing amino acid or not present
  MOD_RES 12: note = Any non-natural amino acid
  MOD_RES 16: note = Any non-natural amino acid
  MOD_RES 17: note = Norleucine
XIIRNIARHLAXVGDXXDR

SEQ ID NO: 46 - protein, 18 aa, synthetic construct
  REGION 1..18: note = Description of Artificial Sequence: Syntheticpeptide
  MOD_RES 1: note = Non-natural electrophile containing amino acid or not present
  MOD_RES 11: note = Any non-natural amino acid
  MOD_RES 15: note = Any non-natural amino acid
  MOD_RES 16: note = Norleucine
XIRNIARHLAXVGDXXDR

SEQ ID NO: 47 - protein, 15 aa, synthetic construct
  REGION 1..15: note = Description of Artificial Sequence: Syntheticpeptide
  MOD_RES 1: note = Non-natural electrophile containing amino acid or not present
  MOD_RES 8: note = Any non-natural amino acid
  MOD_RES 12: note = Any non-natural amino acid
  MOD_RES 13: note = Norleucine
XIARHLAXVGDXXDR

SEQ ID NO: 48 - protein, 14 aa, synthetic construct
  REGION 1..14: note = Description of Artificial Sequence: Syntheticpeptide
  MOD_RES 1: note = Non-natural electrophile containing amino acid or not present
  MOD_RES 7: note = Any non-natural amino acid
  MOD_RES 11: note = Any non-natural amino acid
  MOD_RES 12: note = Norleucine
XARHLAXVGDXXDR

SEQ ID NO: 49 - protein, 16 aa, synthetic construct
  REGION 1..16: note = Description of Artificial Sequence: Syntheticpeptide
  MOD_RES 1: note = Non-natural electrophile containing amino acid or not present
  MOD_RES 2: note = Any non-natural amino acid
  MOD_RES 6: note = Any non-natural amino acid
XXTQLXRFGDKLNFRQ

SEQ ID NO: 50 - protein, 16 aa, synthetic construct
  REGION 1..16: note = Description of Artificial Sequence: Syntheticpeptide
  MOD_RES 1: note = Non-natural electrophile containing amino acid or not present
  MOD_RES 3: note = Any non-natural amino acid
  MOD_RES 7: note = Any non-natural amino acid
XAXQLRXFGDKLNFRQ

SEQ ID NO: 51 - protein, 16 aa, synthetic construct
  REGION 1..16: note = Description of Artificial Sequence: Syntheticpeptide
  MOD_RES 1: note = Non-natural electrophile containing amino acid or not present
  MOD_RES 4: note = Any non-natural amino acid
  MOD_RES 8: note = Any non-natural amino acid
XATXLRRXGDKLNFRQ

SEQ ID NO: 52 - protein, 16 aa, synthetic construct
  REGION 1..16: note = Description of Artificial Sequence: Syntheticpeptide
  MOD_RES 1: note = Non-natural electrophile containing amino acid or not present
  MOD_RES 5: note = Any non-natural amino acid
  MOD_RES 9: note = Any non-natural amino acid
XATQXRRFXDKLNFRQ

SEQ ID NO: 53 - protein, 16 aa, synthetic construct
  REGION 1..16: note = Description of Artificial Sequence: Syntheticpeptide
  MOD_RES 1: note = Non-natural electrophile containing amino acid or not present
  MOD_RES 6: note = Any non-natural amino acid
  MOD_RES 10: note = Any non-natural amino acid
XATQLXRFGXKLNFRQ

SEQ ID NO: 54 - protein, 16 aa, synthetic construct
  REGION 1..16: note = Description of Artificial Sequence: Syntheticpeptide
  MOD_RES 1: note = Non-natural electrophile containing amino acid or not present
  MOD_RES 7: note = Any non-natural amino acid
  MOD_RES 11: note = Any non-natural amino acid
XATQLRXFGDXLNFRQ

SEQ ID NO: 55 - protein, 16 aa, synthetic construct
  REGION 1..16: note = Description of Artificial Sequence: Syntheticpeptide
  MOD_RES 1: note = Non-natural electrophile containing amino acid or not present
  MOD_RES 8: note = Any non-natural amino acid
  MOD_RES 12: note = Any non-natural amino acid
XATQLRRXGDKXNFRQ

SEQ ID NO: 56 - protein, 16 aa, synthetic construct
  REGION 1..16: note = Description of Artificial Sequence: Syntheticpeptide
  MOD_RES 1: note = Non-natural electrophile containing amino acid or not present
  MOD_RES 9: note = Any non-natural amino acid
  MOD_RES 13: note = Any non-natural amino acid
XATQLRRFXDKLXFRQ

SEQ ID NO: 57 - protein, 16 aa, synthetic construct
  REGION 1..16: note = Description of Artificial Sequence: Syntheticpeptide
  MOD_RES 1: note = Non-natural electrophile containing amino acid or not present
  MOD_RES 10: note = Any non-natural amino acid
  MOD_RES 14: note = Any non-natural amino acid
XATQLRRFGXKLNXRQ

SEQ ID NO: 58 - protein, 16 aa, synthetic construct
  REGION 1..16: note = Description of Artificial Sequence: Syntheticpeptide
  MOD_RES 1: note = Non-natural electrophile containing amino acid or not present
  MOD_RES 12: note = Any non-natural amino acid
  MOD_RES 16: note = Any non-natural amino acid
XATQLRRFGDKXNFRX

SEQ ID NO: 59 - protein, 17 aa, synthetic construct
  REGION 1..17: note = Description of Artificial Sequence: Syntheticpeptide
  MOD_RES 1: note = Non-natural electrophile containing amino acid or not present
  MOD_RES 13: note = Any non-natural amino acid
  MOD_RES 17: note = Any non-natural amino acid
XATQLRRFGDKLXFRQX

SEQ ID NO: 60 - protein, 16 aa, synthetic construct
  REGION 1..16: note = Description of Artificial Sequence: Syntheticpeptide
  MOD_RES 1: note = Non-natural electrophile containing amino acid or not present
  MOD_RES 2: note = R-octenyl alanine
  MOD_RES 9: note = Any non-natural amino acid
XATQLRRFXDKLNFRQ

SEQ ID NO: 61 - protein, 16 aa, synthetic construct
  REGION 1..16: note = Description of Artificial Sequence: Syntheticpeptide
  MOD_RES 1: note = Non-natural electrophile containing amino acid or not present
  MOD_RES 3: note = R-octenyl alanine
  MOD_RES 10: note = Any non-natural amino acid
XAAQLRRFGXKLNFRQ

SEQ ID NO: 62 - protein, 16 aa, synthetic construct
  REGION 1..16: note = Description of Artificial Sequence: Syntheticpeptide
  MOD_RES 1: note = Non-natural electrophile containing amino acid or not present
  MOD_RES 4: note = R-octenyl alanine
  MOD_RES 11: note = Any non-natural amino acid
XATXLRRFGDXLNFRQ

SEQ ID NO: 63 - protein, 16 aa, synthetic construct
  REGION 1..16: note = Description of Artificial Sequence: Syntheticpeptide
  MOD_RES 1: note = Non-natural electrophile containing amino acid or not present
  MOD_RES 5: note = R-octenyl alanine
  MOD_RES 12: note = Any non-natural amino acid
XATQARRFGDKXNFRQ

SEQ ID NO: 64 - protein, 16 aa, synthetic construct
  REGION 1..16: note = Description of Artificial Sequence: Syntheticpeptide
  MOD_RES 1: note = Non-natural electrophile containing amino acid or not present
  MOD_RES 6: note = R-octenyl alanine
  MOD_RES 13: note = Any non-natural amino acid
XATQLARFGDKLXFRQ

SEQ ID NO: 65 - protein, 16 aa, synthetic construct
  REGION 1..16: note = Description of Artificial Sequence: Syntheticpeptide
  MOD_RES 1: note = Non-natural electrophile containing amino acid or not present
  MOD_RES 7: note = R-octenyl alanine
  MOD_RES 14: note = Any non-natural amino acid
XATQLRAFGDKLNXRQ

SEQ ID NO: 66 - protein, 16 aa, synthetic construct
  REGION 1..16: note = Description of Artificial Sequence: Syntheticpeptide
  MOD_RES 1: note = Non-natural electrophile containing amino acid or not present
  MOD_RES 8: note = R-octenyl alanine
  MOD_RES 15: note = Any non-natural amino acid
XATQLRRAGDKLNFXQ

SEQ ID NO: 67 - protein, 16 aa, synthetic construct
  REGION 1..16: note = Description of Artificial Sequence: Syntheticpeptide
  MOD_RES 1: note = Non-natural electrophile containing amino acid or not present
  MOD_RES 9: note = R-octenyl alanine
  MOD_RES 16: note = Any non-natural amino acid
XATQLRRFADKLNFRX

SEQ ID NO: 68 - protein, 14 aa, synthetic construct
  REGION 1..14: note = Description of Artificial Sequence: Syntheticpeptide
  MOD_RES 1: note = Non-natural electrophile containing amino acid or not present
  MOD_RES 2: note = Any non-natural amino acid
  MOD_RES 6: note = Any non-natural amino acid
XXRQLXIIGDDINR

SEQ ID NO: 69 - protein, 14 aa, synthetic construct
  REGION 1..14: note = Description of Artificial Sequence: Syntheticpeptide
  MOD_RES 1: note = Non-natural electrophile containing amino acid or not present
  MOD_RES 4: note = Any non-natural amino acid
  MOD_RES 8: note = Any non-natural amino acid
XGRXLAIXGDDINR

SEQ ID NO: 70 - protein, 14 aa, synthetic construct
  REGION 1..14: note = Description of Artificial Sequence: Syntheticpeptide
  MOD_RES 1: note = Non-natural electrophile containing amino acid or not present
  MOD_RES 5: note = Any non-natural amino acid
  MOD_RES 9: note = Any non-natural amino acid
XGRQXAIIXDDINR

SEQ ID NO: 71 - protein, 14 aa, synthetic construct
  REGION 1..14: note = Description of Artificial Sequence: Syntheticpeptide
  MOD_RES 1: note = Non-natural electrophile containing amino acid or not present
  MOD_RES 6: note = Any non-natural amino acid
  MOD_RES 10: note = Any non-natural amino acid
XGRQLXIIGXDINR

SEQ ID NO: 72 - protein, 14 aa, synthetic construct
  REGION 1..14: note = Description of Artificial Sequence: Syntheticpeptide
  MOD_RES 1: note = Non-natural electrophile containing amino acid or not present
  MOD_RES 7: note = Any non-natural amino acid
  MOD_RES 11: note = Any non-natural amino acid
XGRQLAXIGDXINR

SEQ ID NO: 73 - protein, 14 aa, synthetic construct
  REGION 1..14: note = Description of Artificial Sequence: Syntheticpeptide
  MOD_RES 1: note = Non-natural electrophile containing amino acid or not present
  MOD_RES 8: note = Any non-natural amino acid
  MOD_RES 12: note = Any non-natural amino acid
XGRQLAIXGDDXNR

SEQ ID NO: 74 - protein, 14 aa, synthetic construct
  REGION 1..14: note = Description of Artificial Sequence: Syntheticpeptide
  MOD_RES 1: note = Non-natural electrophile containing amino acid or not present
  MOD_RES 9: note = Any non-natural amino acid
  MOD_RES 13: note = Any non-natural amino acid
XGRQLAIIXDDIXR

SEQ ID NO: 75 - protein, 14 aa, synthetic construct
  REGION 1..14: note = Description of Artificial Sequence: Syntheticpeptide
  MOD_RES 1: note = Non-natural electrophile containing amino acid or not present
  MOD_RES 10: note = Any non-natural amino acid
  MOD_RES 14: note = Any non-natural amino acid
XGRQLAIIGXDINX

SEQ ID NO: 76 - protein, 15 aa, synthetic construct
  REGION 1..15: note = Description of Artificial Sequence: Syntheticpeptide
  MOD_RES 1: note = Non-natural electrophile containing amino acid or not present
  MOD_RES 11: note = Any non-natural amino acid
  MOD_RES 15: note = Any non-natural amino acid
XGRQLAIIGDXINRX

SEQ ID NO: 77 - protein, 14 aa, synthetic construct
  REGION 1..14: note = Description of Artificial Sequence: Syntheticpeptide
  MOD_RES 1: note = Non-natural electrophile containing amino acid or not present
  MOD_RES 2: note = R-octenyl alanine
  MOD_RES 9: note = Any non-natural amino acid
XARQLAIIXDDINR

SEQ ID NO: 78 - protein, 14 aa, synthetic construct
  REGION 1..14: note = Description of Artificial Sequence: Syntheticpeptide
  MOD_RES 1: note = Non-natural electrophile containing amino acid or not present
  MOD_RES 3: note = R-octenyl alanine
  MOD_RES 10: note = Any non-natural amino acid
XGAQLAIIGXDINR

SEQ ID NO: 79 - protein, 14 aa, synthetic construct
  REGION 1..14: note = Description of Artificial Sequence: Syntheticpeptide
  MOD_RES 1: note = Non-natural electrophile containing amino acid or not present
  MOD_RES 4: note = R-octenyl alanine
  MOD_RES 11: note = Any non-natural amino acid
XGRALAIIGDXINR

SEQ ID NO: 80 - protein, 14 aa, synthetic construct
  REGION 1..14: note = Description of Artificial Sequence: Syntheticpeptide
  MOD_RES 1: note = Non-natural electrophile containing amino acid or not present
  MOD_RES 5: note = R-octenyl alanine
  MOD_RES 12: note = Any non-natural amino acid
XGRQAAIIGDDXNR

SEQ ID NO: 81 - protein, 14 aa, synthetic construct
  REGION 1..14: note = Description of Artificial Sequence: Syntheticpeptide
  MOD_RES 1: note = Non-natural electrophile containing amino acid or not present
  MOD_RES 6: note = R-octenyl alanine
  MOD_RES 13: note = Any non-natural amino acid
XGRQLAIIGDDIXR

SEQ ID NO: 82 - protein, 14 aa, synthetic construct
  REGION 1..14: note = Description of Artificial Sequence: Syntheticpeptide
  MOD_RES 1: note = Non-natural electrophile containing amino acid or not present
  MOD_RES 7: note = R-octenyl alanine
  MOD_RES 14: note = Any non-natural amino acid
XGRQLAAIGDDINX

SEQ ID NO: 83 - protein, 15 aa, synthetic construct
  REGION 1..15: note = Description of Artificial Sequence: Syntheticpeptide
  MOD_RES 1: note = Non-natural electrophile containing amino acid or not present
  MOD_RES 8: note = R-octenyl alanine
  MOD_RES 15: note = Any non-natural amino acid
XGRQLAIAGDDINRX

SEQ ID NO: 84 - protein, 15 aa, synthetic construct
  REGION 1..15: note = Description of Artificial Sequence: Syntheticpeptide
  MOD_RES 1: note = Non-natural electrophile containing amino acid or not present
  MOD_RES 3: note = Any non-natural amino acid
  MOD_RES 7: note = Any non-natural amino acid
XVXRQLXIIGDDINR

SEQ ID NO: 85 - protein, 15 aa, synthetic construct
  REGION 1..15: note = Description of Artificial Sequence: Syntheticpeptide
  MOD_RES 1: note = Non-natural electrophile containing amino acid or not present
  MOD_RES 4: note = Any non-natural amino acid
  MOD_RES 8: note = Any non-natural amino acid
XVGXQLAXIGDDINR

SEQ ID NO: 86 - protein, 15 aa, synthetic construct
  REGION 1..15: note = Description of Artificial Sequence: Syntheticpeptide
  MOD_RES 1: note = Non-natural electrophile containing amino acid or not present
  MOD_RES 5: note = Any non-natural amino acid
  MOD_RES 9: note = Any non-natural amino acid
XVGRXLAIXGDDINR

SEQ ID NO: 87 - protein, 15 aa, synthetic construct
  REGION 1..15: note = Description of Artificial Sequence: Syntheticpeptide
  MOD_RES 1: note = Non-natural electrophile containing amino acid or not present
  MOD_RES 6: note = Any non-natural amino acid
  MOD_RES 10: note = Any non-natural amino acid
XVGRQXAIIXDDINR

SEQ ID NO: 88 - protein, 15 aa, synthetic construct
  REGION 1..15: note = Description of Artificial Sequence: Syntheticpeptide
  MOD_RES 1: note = Non-natural electrophile containing amino acid or not present
  MOD_RES 7: note = Any non-natural amino acid
  MOD_RES 11: note = Any non-natural amino acid
XVGRQLXIIGXDINR

SEQ ID NO: 89 - protein, 15 aa, synthetic construct
  REGION 1..15: note = Description of Artificial Sequence: Syntheticpeptide
  MOD_RES 1: note = Non-natural electrophile containing amino acid or not present
  MOD_RES 8: note = Any non-natural amino acid
  MOD_RES 12: note = Any non-natural amino acid
XVGRQLAXIGDXINR

SEQ ID NO: 90 - protein, 15 aa, synthetic construct
  REGION 1..15: note = Description of Artificial Sequence: Syntheticpeptide
  MOD_RES 1: note = Non-natural electrophile containing amino acid or not present
  MOD_RES 9: note = Any non-natural amino acid
  MOD_RES 13: note = Any non-natural amino acid
XVGRQLAIXGDDXNR

SEQ ID NO: 91 - protein, 15 aa, synthetic construct
  REGION 1..15: note = Description of Artificial Sequence: Syntheticpeptide
  MOD_RES 1: note = Non-natural electrophile containing amino acid or not present
  MOD_RES 10: note = Any non-natural amino acid
  MOD_RES 14: note = Any non-natural amino acid
XVGRQLAIIXDDIXR

SEQ ID NO: 92 - protein, 15 aa, synthetic construct
  REGION 1..15: note = Description of Artificial Sequence: Syntheticpeptide
  MOD_RES 1: note = Non-natural electrophile containing amino acid or not present
  MOD_RES 11: note = Any non-natural amino acid
  MOD_RES 15: note = Any non-natural amino acid
XVGRQLAIIGXDINX

SEQ ID NO: 93 - protein, 16 aa, synthetic construct
  REGION 1..16: note = Description of Artificial Sequence: Syntheticpeptide
  MOD_RES 1: note = Non-natural electrophile containing amino acid or not present
  MOD_RES 12: note = Any non-natural amino acid
  MOD_RES 16: note = Any non-natural amino acid
XVGRQLAIIGDXINRX

SEQ ID NO: 94 - protein, 15 aa, synthetic construct
  REGION 1..15: note = Description of Artificial Sequence: Syntheticpeptide
  MOD_RES 1: note = Non-natural electrophile containing amino acid or not present
  MOD_RES 3: note = R-octenyl alanine
  MOD_RES 10: note = Any non-natural amino acid
XVARQLAIIXDDINR

SEQ ID NO: 95 - protein, 15 aa, synthetic construct
  REGION 1..15: note = Description of Artificial Sequence: Syntheticpeptide
  MOD_RES 1: note = Non-natural electrophile containing amino acid or not present
  MOD_RES 4: note = R-octenyl alanine
  MOD_RES 11: note = Any non-natural amino acid
XVGAQLAIIGXDINR

SEQ ID NO: 96 - protein, 15 aa, synthetic construct
  REGION 1..15: note = Description of Artificial Sequence: Syntheticpeptide
  MOD_RES 1: note = Non-natural electrophile containing amino acid or not present
  MOD_RES 5: note = R-octenyl alanine
  MOD_RES 12: note = Any non-natural amino acid
XVGRALAIIGDXINR

SEQ ID NO: 97 - protein, 15 aa, synthetic construct
  REGION 1..15: note = Description of Artificial Sequence: Syntheticpeptide
  MOD_RES 1: note = Non-natural electrophile containing amino acid or not present
  MOD_RES 6: note = R-octenyl alanine
  MOD_RES 13: note = Any non-natural amino acid
XVGRQAAIIGDDXNR

SEQ ID NO: 98 - protein, 15 aa, synthetic construct
  REGION 1..15: note = Description of Artificial Sequence: Syntheticpeptide
  MOD_RES 1: note = Non-natural electrophile containing amino acid or not present
  MOD_RES 7: note = R-octenyl alanine
  MOD_RES 14: note = Any non-natural amino acid
XVGRQLAIIGDDIXR

SEQ ID NO: 99 - protein, 15 aa, synthetic construct
  REGION 1..15: note = Description of Artificial Sequence: Syntheticpeptide
  MOD_RES 1: note = Non-natural electrophile containing amino acid or not present
  MOD_RES 8: note = R-octenyl alanine
  MOD_RES 15: note = Any non-natural amino acid
XVGRQLAAIGDDINX

SEQ ID NO: 100 - protein, 16 aa, synthetic construct
  REGION 1..16: note = Description of Artificial Sequence: Syntheticpeptide
  MOD_RES 1: note = Non-natural electrophile containing amino acid or not present
  MOD_RES 9: note = R-octenyl alanine
  MOD_RES 16: note = Any non-natural amino acid
XVGRQLAIAGDDINRX

SEQ ID NO: 101 - protein, 15 aa, synthetic construct
  REGION 1..15: note = Description of Artificial Sequence: Syntheticpeptide
  MOD_RES 1: note = Non-natural electrophile containing amino acid or not present
  MOD_RES 2: note = Any non-natural amino acid
  MOD_RES 6: note = Any non-natural amino acid
XXSESXKRIGDELDS

SEQ ID NO: 102 - protein, 15 aa, synthetic construct
  REGION 1..15: note = Description of Artificial Sequence: Syntheticpeptide
  MOD_RES 1: note = Non-natural electrophile containing amino acid or not present
  MOD_RES 3: note = Any non-natural amino acid
  MOD_RES 7: note = Any non-natural amino acid
XLXESLXRIGDELDS

SEQ ID NO: 103 - protein, 15 aa, synthetic construct
  REGION 1..15: note = Description of Artificial Sequence: Syntheticpeptide
  MOD_RES 1: note = Non-natural electrophile containing amino acid or not present
  MOD_RES 4: note = Any non-natural amino acid
  MOD_RES 8: note = Any non-natural amino acid
XLSXSLKXIGDELDS

SEQ ID NO: 104 - protein, 15 aa, synthetic construct
  REGION 1..15: note = Description of Artificial Sequence: Syntheticpeptide
  MOD_RES 1: note = Non-natural electrophile containing amino acid or not present
  MOD_RES 5: note = Any non-natural amino acid
  MOD_RES 9: note = Any non-natural amino acid
XLSEXLKRXGDELDS

SEQ ID NO: 105 - protein, 15 aa, synthetic construct
  REGION 1..15: note = Description of Artificial Sequence: Syntheticpeptide
  MOD_RES 1: note = Non-natural electrophile containing amino acid or not present
  MOD_RES 6: note = Any non-natural amino acid
  MOD_RES 10: note = Any non-natural amino acid
XLSESXKRIXDELDS

SEQ ID NO: 106 - protein, 15 aa, synthetic construct
  REGION 1..15: note = Description of Artificial Sequence: Syntheticpeptide
  MOD_RES 1: note = Non-natural electrophile containing amino acid or not present
  MOD_RES 7: note = Any non-natural amino acid
  MOD_RES 11: note = Any non-natural amino acid
XLSESLXRIGXELDS

SEQ ID NO: 107 - protein, 15 aa, synthetic construct
  REGION 1..15: note = Description of Artificial Sequence: Syntheticpeptide
  MOD_RES 1: note = Non-natural electrophile containing amino acid or not present
  MOD_RES 8: note = Any non-natural amino acid
  MOD_RES 12: note = Any non-natural amino acid
XLSESLKXIGDXLDS

SEQ ID NO: 108 - protein, 15 aa, synthetic construct
  REGION 1..15: note = Description of Artificial Sequence: Syntheticpeptide
  MOD_RES 1: note = Non-natural electrophile containing amino acid or not present
  MOD_RES 9: note = Any non-natural amino acid
  MOD_RES 13: note = Any non-natural amino acid
XLSESLKRXGDEXDS

SEQ ID NO: 109 - protein, 15 aa, synthetic construct
  REGION 1..15: note = Description of Artificial Sequence: Syntheticpeptide
  MOD_RES 1: note = Non-natural electrophile containing amino acid or not present
  MOD_RES 10: note = Any non-natural amino acid
  MOD_RES 14: note = Any non-natural amino acid
XLSESLKRIXDELXS

SEQ ID NO: 110 - protein, 15 aa, synthetic construct
  REGION 1..15: note = Description of Artificial Sequence: Syntheticpeptide
  MOD_RES 1: note = Non-natural electrophile containing amino acid or not present
  MOD_RES 11: note = Any non-natural amino acid
  MOD_RES 15: note = Any non-natural amino acid
XLSESLKRIGXELDX

SEQ ID NO: 111 - protein, 16 aa, synthetic construct
  REGION 1..16: note = Description of Artificial Sequence: Syntheticpeptide
  MOD_RES 1: note = Non-natural electrophile containing amino acid or not present
  MOD_RES 12: note = Any non-natural amino acid
  MOD_RES 16: note = Any non-natural amino acid
XLSESLKRIGDXLDSX

SEQ ID NO: 112 - protein, 15 aa, synthetic construct
  REGION 1..15: note = Description of Artificial Sequence: Syntheticpeptide
  MOD_RES 1: note = Non-natural electrophile containing amino acid or not present
  MOD_RES 2: note = R-octenyl alanine
  MOD_RES 9: note = Any non-natural amino acid
XASESLKRXGDELDS

SEQ ID NO: 113 - protein, 15 aa, synthetic construct
  REGION 1..15: note = Description of Artificial Sequence: Syntheticpeptide
  MOD_RES 1: note = Non-natural electrophile containing amino acid or not present
  MOD_RES 3: note = R-octenyl alanine
  MOD_RES 10: note = Any non-natural amino acid
XLAESLKRIXDELDS

SEQ ID NO: 114 - protein, 15 aa, synthetic construct
  REGION 1..15: note = Description of Artificial Sequence: Syntheticpeptide
  MOD_RES 1: note = Non-natural electrophile containing amino acid or not present
  MOD_RES 4: note = R-octenyl alanine
  MOD_RES 11: note = Any non-natural amino acid
XLSASLKRIGXELDS

SEQ ID NO: 115 - protein, 15 aa, synthetic construct
  REGION 1..15: note = Description of Artificial Sequence: Syntheticpeptide
  MOD_RES 1: note = Non-natural electrophile containing amino acid or not present
  MOD_RES 5: note = R-octenyl alanine
  MOD_RES 12: note = Any non-natural amino acid
XLSEALKRIGDXLDS

SEQ ID NO: 116 - protein, 15 aa, synthetic construct
  REGION 1..15: note = Description of Artificial Sequence: Syntheticpeptide
  MOD_RES 1: note = Non-natural electrophile containing amino acid or not present
  MOD_RES 6: note = R-octenyl alanine
  MOD_RES 13: note = Any non-natural amino acid
XLSESAKRIGDEXDS

SEQ ID NO: 117 - protein, 15 aa, synthetic construct
  REGION 1..15: note = Description of Artificial Sequence: Syntheticpeptide
  MOD_RES 1: note = Non-natural electrophile containing amino acid or not present
  MOD_RES 7: note = R-octenyl alanine
  MOD_RES 14: note = Any non-natural amino acid
XLSESLARIGDELXS

SEQ ID NO: 118 - protein, 15 aa, synthetic construct
  REGION 1..15: note = Description of Artificial Sequence: Syntheticpeptide
  MOD_RES 1: note = Non-natural electrophile containing amino acid or not present
  MOD_RES 8: note = R-octenyl alanine
  MOD_RES 15: note = Any non-natural amino acid
XLSESLKAIGDELDX

SEQ ID NO: 119 - protein, 16 aa, synthetic construct
  REGION 1..16: note = Description of Artificial Sequence: Syntheticpeptide
  MOD_RES 1: note = Non-natural electrophile containing amino acid or not present
  MOD_RES 9: note = R-octenyl alanine
  MOD_RES 16: note = Any non-natural amino acid
XLSESLKRAGDELDSX

SEQ ID NO: 120 - skipped

SEQ ID NO: 121 - protein, 15 aa, synthetic construct
  REGION 1..15: note = Description of Artificial Sequence: Syntheticpeptide
ATQLRRFGDKLNFRQ

SEQ ID NO: 122 - protein, 26 aa, synthetic construct
  REGION 1..26: note = Description of Artificial Sequence: Syntheticpeptide
AELEVECATQLRRFGDKLNFRQKLLN

SEQ ID NO: 123 - protein, 22 aa, synthetic construct
  REGION 1..22: note = Description of Artificial Sequence: Syntheticpeptide
EIWIAQELRRIGDEFNAYYARR

SEQ ID NO: 124 - protein, 21 aa, synthetic construct
  REGION 1..21: note = Description of Artificial Sequence: Syntheticpeptide
DIIRNIARHLAQVGDSMDRSI

SEQ ID NO: 125 - protein, 22 aa, synthetic construct
  REGION 1..22: note = Description of Artificial Sequence: Syntheticpeptide
SSTMGQVGRQLAIIGDDINRRY

SEQ ID NO: 126 - protein, 25 aa, synthetic construct
  REGION 1..25: note = Description of Artificial Sequence: Syntheticpeptide
QDASTKKLSESLKRIGDELDSNMEL

SEQ ID NO: 127 - protein, 20 aa, synthetic construct
  REGION 1..20: note = Description of Artificial Sequence: Syntheticpeptide
RLAEVCAVLLRLGDELEMIR

SEQ ID NO: 128 - protein, 19 aa, synthetic construct
  REGION 1..19: note = Description of Artificial Sequence: Syntheticpeptide
  MOD_RES 1: note = Non-natural electrophile containing amino acid or not present
XATQLRRFGDKLNFRQKLL

SEQ ID NO: 129 - protein, 23 aa, synthetic construct
  REGION 1..23: note = Description of Artificial Sequence: Syntheticpeptide
  MOD_RES 1: note = Non-natural electrophile containing amino acid or not present
XEVESATQLRRFGDKLNFRQKLL

SEQ ID NO: 130 - protein, 20 aa, synthetic construct
  REGION 1..20: note = Description of Artificial Sequence: Syntheticpeptide
  MOD_RES 1: note = Non-natural electrophile containing amino acid or not present
XIAQELRRIGDEFNAYYARR

SEQ ID NO: 131 - protein, 15 aa, synthetic construct
  REGION 1..15: note = Description of Artificial Sequence: Syntheticpeptide
ATQLRRFGDKLNFRQ

SEQ ID NO: 132 - protein, 19 aa, synthetic construct
  REGION 1..19: note = Description of Artificial Sequence: Syntheticpeptide
IAQELRRIGDEFNAYYARR

SEQ ID NO: 133 - protein, 13 aa, synthetic construct
  REGION 1..13: note = Description of Artificial Sequence: Syntheticpeptide
ARHLAQVGDSMDR

SEQ ID NO: 134 - protein, 13 aa, synthetic construct
  REGION 1..13: note = Description of Artificial Sequence: Syntheticpeptide
GRQLAIIGDDINR

SEQ ID NO: 135 - protein, 14 aa, synthetic construct
  REGION 1..14: note = Description of Artificial Sequence: Syntheticpeptide
LSESLKRIGDELDS

SEQ ID NO: 136 - protein, 13 aa, synthetic construct
  REGION 1..13: note = Description of Artificial Sequence: Syntheticpeptide
CAVLLRLGDELEM

SEQ ID NO: 137 - protein, 10 aa, synthetic construct
  REGION 1..10: note = Description of Artificial Sequence: Syntheticpeptide
  MOD_RES 1: note = Non-natural electrophile containing amino acid
XEVESATQLR

SEQ ID NO: 138 - protein, 6 aa, synthetic construct
  REGION 1..6: note = Description of Artificial Sequence: Syntheticpeptide
  MOD_RES 1: note = Non-natural electrophile containing amino acid
XATQLR

SEQ ID NO: 139 - protein, 9 aa, synthetic construct
  REGION 1..9: note = Description of Artificial Sequence: Syntheticpeptide
  MOD_RES 1: note = Non-natural electrophile containing amino acid
XVESATQLR

SEQ ID NO: 140 - protein, 8 aa, synthetic construct
  REGION 1..8: note = Description of Artificial Sequence: Syntheticpeptide
  MOD_RES 1: note = Non-natural electrophile containing amino acid
XESATQLR

SEQ ID NO: 141 - protein, 7 aa, synthetic construct
  REGION 1..7: note = Description of Artificial Sequence: Syntheticpeptide
  MOD_RES 1: note = Non-natural electrophile containing amino acid
XSATQLR

SEQ ID NO: 142 - protein, 5 aa, synthetic construct
  REGION 1..5: note = Description of Artificial Sequence: Syntheticpeptide
  MOD_RES 5: note = Any cell permeability enhancing amino acid (e.g., amino acidsthat change or shift the distribution of charge or hydrophobiccharacter) or a stability enhancing amino acid (e.g., non-native, D, or alpha methyl amino acid point mutations)
LNFRX

SEQ ID NO: 143 - protein, 6 aa, synthetic construct
  REGION 1..6: note = Description of Artificial Sequence: Syntheticpeptide
  MOD_RES 6: note = Any cell permeability enhancing amino acid (e.g., amino acidsthat change or shift the distribution of charge or hydrophobiccharacter) or a stability enhancing amino acid (e.g., non-native, D, or alpha methyl amino acid point mutations)
LNFRQX

SEQ ID NO: 144 - protein, 7 aa, synthetic construct
  REGION 1..7: note = Description of Artificial Sequence: Syntheticpeptide
  MOD_RES 7: note = Any cell permeability enhancing amino acid (e.g., amino acidsthat change or shift the distribution of charge or hydrophobiccharacter) or a stability enhancing amino acid (e.g., non-native, D, or alpha methyl amino acid point mutations)
LNFRQKX

SEQ ID NO: 145 - protein, 9 aa, synthetic construct
  REGION 1..9: note = Description of Artificial Sequence: Syntheticpeptide
  MOD_RES 9: note = Any cell permeability enhancing amino acid (e.g., amino acidsthat change or shift the distribution of charge or hydrophobiccharacter) or a stability enhancing amino acid (e.g., non-native, D, or alpha methyl amino acid point mutations)
LNFRQKLLX

SEQ ID NO: 146 - protein, 10 aa, synthetic construct
  REGION 1..10: note = Description of Artificial Sequence: Syntheticpeptide
  MOD_RES 10: note = Any cell permeability enhancing amino acid (e.g., amino acidsthat change or shift the distribution of charge or hydrophobiccharacter) or a stability enhancing amino acid (e.g., non-native, D, or alpha methyl amino acid point mutations)
LNFRQKLLKX

SEQ ID NO: 147 - protein, 7 aa, synthetic construct
  REGION 1..7: note = Description of Artificial Sequence: Syntheticpeptide
  MOD_RES 1: note = Non-natural electrophile containing amino acid
XIAQELR

SEQ ID NO: 148 - protein, 6 aa, synthetic construct
  REGION 1..6: note = Description of Artificial Sequence: Syntheticpeptide
  MOD_RES 1: note = Non-natural electrophile containing amino acid
XAQELR

SEQ ID NO: 149 - protein, 7 aa, synthetic construct
  REGION 1..7: note = Description of Artificial Sequence: Syntheticpeptide
  MOD_RES 1: note = Non-natural electrophile containing amino acid
XAQELRR

SEQ ID NO: 150 - protein, 9 aa, synthetic construct
  REGION 1..9: note = Description of Artificial Sequence: Syntheticpeptide
  MOD_RES 9: note = Any cell permeability enhancing amino acid (e.g., amino acidsthat change or shift the distribution of charge or hydrophobiccharacter) or a stability enhancing amino acid (e.g., non-native, D, or alpha methyl amino acid point mutations)
FNAYYARKX

SEQ ID NO: 151 - protein, 9 aa, synthetic construct
  REGION 1..9: note = Description of Artificial Sequence: Syntheticpeptide
  MOD_RES 9: note = Any cell permeability enhancing amino acid (e.g., amino acidsthat change or shift the distribution of charge or hydrophobiccharacter) or a stability enhancing amino acid (e.g., non-native, D, or alpha methyl amino acid point mutations)
FNAYYARRX

SEQ ID NO: 152 - protein, 7 aa, synthetic construct
  REGION 1..7: note = Description of Artificial Sequence: Syntheticpeptide
  MOD_RES 1: note = Non-natural electrophile containing amino acid
XLSESLK

SEQ ID NO: 153 - protein, 6 aa, synthetic construct
  REGION 1..6: note = Description of Artificial Sequence: Syntheticpeptide
  MOD_RES 1: note = Non-natural electrophile containing amino acid
XSESLK

SEQ ID NO: 154 - protein, 6 aa, synthetic construct
  REGION 1..6: note = Description of Artificial Sequence: Syntheticpeptide
  MOD_RES 6: note = Any cell permeability enhancing amino acid (e.g., amino acidsthat change or shift the distribution of charge or hydrophobiccharacter) or a stability enhancing amino acid (e.g., non-native, D, or alpha methyl amino acid point mutations)
LDSNKX

SEQ ID NO: 155 - protein, 5 aa, synthetic construct
  REGION 1..5: note = Description of Artificial Sequence: Syntheticpeptide
  MOD_RES 5: note = Any cell permeability enhancing amino acid (e.g., amino acidsthat change or shift the distribution of charge or hydrophobiccharacter) or a stability enhancing amino acid (e.g., non-native, D, or alpha methyl amino acid point mutations)
LDSNX

SEQ ID NO: 156 - protein, 9 aa, synthetic construct
  REGION 1..9: note = Description of Artificial Sequence: Syntheticpeptide
  MOD_RES 9: note = Any cell permeability enhancing amino acid (e.g., amino acidsthat change or shift the distribution of charge or hydrophobiccharacter) or a stability enhancing amino acid (e.g., non-native, D, or alpha methyl amino acid point mutations)
IGDDINRRX

SEQ ID NO: 157 - protein, 8 aa, synthetic construct
  REGION 1..8: note = Description of Artificial Sequence: Syntheticpeptide
  MOD_RES 8: note = Any cell permeability enhancing amino acid (e.g., amino acidsthat change or shift the distribution of charge or hydrophobiccharacter) or a stability enhancing amino acid (e.g., non-native, D, or alpha methyl amino acid point mutations)
IGDDINRX

SEQ ID NO: 158 - protein, 15 aa, synthetic construct
  REGION 1..15: note = Description of Artificial Sequence: Syntheticpeptide
  MOD_RES 1: note = Non-natural electrophile containing amino acid
XPGGRLAEVCTVLLR

SEQ ID NO: 159 - protein, 14 aa, synthetic construct
  REGION 1..14: note = Description of Artificial Sequence: Syntheticpeptide
  MOD_RES 1: note = Non-natural electrophile containing amino acid
XGGRLAEVCTVLLR

SEQ ID NO: 160 - protein, 9 aa, synthetic construct
  REGION 1..9: note = Description of Artificial Sequence: Syntheticpeptide
  MOD_RES 9: note = Any cell permeability enhancing amino acid (e.g., amino acidsthat change or shift the distribution of charge or hydrophobiccharacter) or a stability enhancing amino acid (e.g., non-native, D, or alpha methyl amino acid point mutations)
ELEQIRPSX

SEQ ID NO: 161 - protein, 7 aa, synthetic construct
  REGION 1..7: note = Description of Artificial Sequence: Syntheticpeptide
  MOD_RES 7: note = Any cell permeability enhancing amino acid (e.g., amino acidsthat change or shift the distribution of charge or hydrophobiccharacter) or a stability enhancing amino acid (e.g., non-native, D, or alpha methyl amino acid point mutations)
ELEQIRX

SEQ ID NO: 162 - protein, 12 aa, synthetic construct
  REGION 1..12: note = Description of Artificial Sequence: Syntheticpeptide
  MOD_RES 1: note = Non-natural electrophile containing amino acid
XDIIRNIARHLA

SEQ ID NO: 163 - protein, 11 aa, synthetic construct
  REGION 1..11: note = Description of Artificial Sequence: Syntheticpeptide
  MOD_RES 1: note = Non-natural electrophile containing amino acid
XIIRNIARHLA

SEQ ID NO: 164 - protein, 6 aa, synthetic construct
  REGION 1..6: note = Description of Artificial Sequence: Syntheticpeptide
  MOD_RES 1: note = Norleucine
  MOD_RES 6: note = Any cell permeability enhancing amino acid (e.g., amino acidsthat change or shift the distribution of charge or hydrophobiccharacter) or a stability enhancing amino acid (e.g., non-native, D, or alpha methyl amino acid point mutations)
XDRSIX

SEQ ID NO: 165 - protein, 7 aa, synthetic construct
  REGION 1..7: note = Description of Artificial Sequence: Syntheticpeptide
  MOD_RES 1: note = Norleucine
  MOD_RES 7: note = Any cell permeability enhancing amino acid (e.g., amino acidsthat change or shift the distribution of charge or hydrophobiccharacter) or a stability enhancing amino acid (e.g., non-native, D, or alpha methyl amino acid point mutations)
XDRSIRX

SEQ ID NO: 166 - protein, 13 aa, synthetic construct
  REGION 1..13: note = Description of Artificial Sequence: Syntheticpeptide
  MOD_RES 1: note = Non-natural electrophile containing amino acid
XEQWAREIGAQLR

SEQ ID NO: 167 - protein, 12 aa, synthetic construct
  REGION 1..12: note = Description of Artificial Sequence: Syntheticpeptide
  MOD_RES 1: note = Non-natural electrophile containing amino acid
XQWAREIGAQLR

SEQ ID NO: 168 - protein, 9 aa, synthetic construct
  REGION 1..9: note = Description of Artificial Sequence: Syntheticpeptide
  MOD_RES 1: note = Non-natural electrophile containing amino acid
XREIGAQLR

SEQ ID NO: 169 - protein, 8 aa, synthetic construct
  REGION 1..8: note = Description of Artificial Sequence: Syntheticpeptide
  MOD_RES 1: note = Non-natural electrophile containing amino acid
XEIGAQLR

SEQ ID NO: 170 - protein, 6 aa, synthetic construct
  REGION 1..6: note = Description of Artificial Sequence: Syntheticpeptide
  MOD_RES 6: note = Any cell permeability enhancing amino acid (e.g., amino acidsthat change or shift the distribution of charge or hydrophobiccharacter) or a stability enhancing amino acid (e.g., non-native, D, or alpha methyl amino acid point mutations)
LNAQYX

SEQ ID NO: 171 - protein, 7 aa, synthetic construct
  REGION 1..7: note = Description of Artificial Sequence: Syntheticpeptide
  MOD_RES 7: note = Any cell permeability enhancing amino acid (e.g., amino acidsthat change or shift the distribution of charge or hydrophobiccharacter) or a stability enhancing amino acid (e.g., non-native, D, or alpha methyl amino acid point mutations)
LNAQYEX

SEQ ID NO: 172 - protein, 8 aa, synthetic construct
  REGION 1..8: note = Description of Artificial Sequence: Syntheticpeptide
  MOD_RES 8: note = Any cell permeability enhancing amino acid (e.g., amino acidsthat change or shift the distribution of charge or hydrophobiccharacter) or a stability enhancing amino acid (e.g., non-native, D, or alpha methyl amino acid point mutations)
LNFRQKLX

SEQ ID NO: 173 - protein, 25 aa, synthetic construct
  REGION 1..25: note = Description of Artificial Sequence: Syntheticpeptide
  MOD_RES 1: note = Non-natural electrophile containing amino acid
  REGION 2..5: note = MISC_FEATURE - May or may not be present
  REGION 2..10: note = MISC_FEATURE - This region may encompass "EVESATQLR" or "VESATQLR"or "ESATQLR" or "SATQLR" or "ATQLR" wherein somepositions may be absent
  MOD_RES 11: note = Any amino acid
  MOD_RES 15: note = Any amino acid
  REGION 16..24: note = MISC_FEATURE - This region may encompass "LNFRQKLLK" or "LNFRQKLL"or "LNFRQKL" or "LNFRQK" or "LNFRQ" or "LNFR"wherein some positions may be absent
  REGION 20..24: note = MISC_FEATURE - May or may not be present
  MOD_RES 25: note = Any cell permeability enhancing amino acid (e.g., amino acidsthat change or shift the distribution of charge or hydrophobiccharacter) or a stability enhancing amino acid (e.g., non-native, D, or alpha methyl amino acid point mutations)
  REGION 1..25: note = See specification as filed for detailed description ofsubstitutions and preferred embodiments
XEVESATQLRXFGDXLNFRQKLLKX

SEQ ID NO: 174 - protein, 22 aa, synthetic construct
  REGION 1..22: note = Description of Artificial Sequence: Syntheticpeptide
  MOD_RES 1: note = Non-natural electrophile containing amino acid
  SITE 2: note = MISC_FEATURE - May or may not be present
  REGION 2..8: note = MISC_FEATURE - This region may encompass "IAQELR" or "AQELR"or "AQELRR" wherein some positions may be absent
  SITE 8: note = MISC_FEATURE - May or may not be present
  MOD_RES 9: note = Any amino acid
  MOD_RES 13: note = Any amino acid
  REGION 14..21: note = MISC_FEATURE - This region may encompass "FNAYYARK" or "FNAYYARR"wherein some positions may be absent
  MOD_RES 21: note = Arg or Lys
  MOD_RES 22: note = Any cell permeability enhancing amino acid (e.g., amino acidsthat change or shift the distribution of charge or hydrophobiccharacter) or a stability enhancing amino acid (e.g., non-native, D, or alpha methyl amino acid point mutations)
  REGION 1..22: note = See specification as filed for detailed description ofsubstitutions and preferred embodiments
XIAQELRRXIGDXFNAYYARXX

SEQ ID NO: 175 - protein, 18 aa, synthetic construct
  REGION 1..18: note = Description of Artificial Sequence: Syntheticpeptide
  MOD_RES 1: note = Non-natural electrophile containing amino acid
  SITE 2: note = MISC_FEATURE - May or may not be present
  REGION 2..7: note = MISC_FEATURE - This region may encompass "LSESLK" or "SESLK"wherein some positions may be absent
  MOD_RES 8: note = Any amino acid
  MOD_RES 12: note = Any amino acid
  REGION 13..17: note = MISC_FEATURE - This region may encompass "LDSNK" or "LDSN"wherein some positions may be absent
  SITE 17: note = MISC_FEATURE - May or may not be present
  MOD_RES 18: note = Any cell permeability enhancing amino acid (e.g., amino acidsthat change or shift the distribution of charge or hydrophobiccharacter) or a stability enhancing amino acid (e.g., non-native, D, or alpha methyl amino acid point mutations)
  REGION 1..18: note = See specification as filed for detailed description ofsubstitutions and preferred embodiments
XLSESLKXIGDXLDSNKX

SEQ ID NO: 176 - protein, 17 aa, synthetic construct
  REGION 1..17: note = Description of Artificial Sequence: Syntheticpeptide
  MOD_RES 1: note = Non-natural electrophile containing amino acid
  SITE 2: note = MISC_FEATURE - May or may not be present
  REGION 2..3: note = MISC_FEATURE - This region may encompass "VG" or "G"wherein some positions may be absent
  MOD_RES 4: note = Any amino acid
  MOD_RES 8: note = Any amino acid
  REGION 9..16: note = MISC_FEATURE - This region may encompass "IGDDINRR" or "IGDDINR"wherein some positions may be absent
  SITE 16: note = MISC_FEATURE - May or may not be present
  MOD_RES 17: note = Any cell permeability enhancing amino acid (e.g., amino acidsthat change or shift the distribution of charge or hydrophobiccharacter) or a stability enhancing amino acid (e.g., non-native, D, or alpha methyl amino acid point mutations)
  REGION 1..17: note = See specification as filed for detailed description ofsubstitutions and preferred embodiments
XVGXQLAXIGDDINRRX

SEQ ID NO: 177 - protein, 29 aa, synthetic construct
  REGION 1..29: note = Description of Artificial Sequence: Syntheticpeptide
  MOD_RES 1: note = Non-natural electrophile containing amino acid
  SITE 2: note = MISC_FEATURE - May or may not be present
  REGION 2..15: note = MISC_FEATURE - This region may encompass "PGGRLAEVCTVLLR" or"GGRLAEVCTVLLR" wherein some positions may be absent
  MOD_RES 16: note = Any amino acid
  MOD_RES 20: note = Any amino acid
  REGION 21..28: note = MISC_FEATURE - This region may encompass "ELEQIRPS" or "ELEQIR"wherein some positions may be absent
  REGION 27..28: note = MISC_FEATURE - May or may not be present
  MOD_RES 29: note = Any cell permeability enhancing amino acid (e.g., amino acidsthat change or shift the distribution of charge or hydrophobiccharacter) or a stability enhancing amino acid (e.g., non-native, D, or alpha methyl amino acid point mutations)
  REGION 1..29: note = See specification as filed for detailed description ofsubstitutions and preferred embodiments
XPGGRLAEVCTVLLRXLGDXELEQIRPSX

SEQ ID NO: 178 - protein, 24 aa, synthetic construct
  REGION 1..24: note = Description of Artificial Sequence: Syntheticpeptide
  MOD_RES 1: note = Non-natural electrophile containing amino acid
  SITE 2: note = MISC_FEATURE - May or may not be present
  REGION 2..12: note = MISC_FEATURE - This region may encompass "DIIRNIARHLA" or "IIRNIARHLA"wherein some positions may be absent
  MOD_RES 13: note = Any amino acid
  MOD_RES 17: note = Any amino acid
  MOD_RES 18: note = Norleucine
  REGION 18..23: note = MISC_FEATURE - This region may encompass "BDRSIR" or "BDRSI" wherein B isnorleucine and some positions may be absent
  SITE 23: note = MISC_FEATURE - May or may not be present
  MOD_RES 24: note = Any cell permeability enhancing amino acid (e.g., amino acidsthat change or shift the distribution of charge or hydrophobiccharacter) or a stability enhancing amino acid (e.g., non-native, D, or alpha methyl amino acid point mutations)
  REGION 1..24: note = See specification as filed for detailed description ofsubstitutions and preferred embodiments
XDIIRNIARHLAXVGDXXDRSIRX

SEQ ID NO: 179 - protein, 25 aa, synthetic construct
  REGION 1..25: note = Description of Artificial Sequence: Syntheticpeptide
  MOD_RES 1: note = Non-natural electrophile containing amino acid
  REGION 2..6: note = MISC_FEATURE - May or may not be present
  REGION 2..13: note = MISC_FEATURE - This region may encompass "EQWAREIGAQLR" or "QWAREIGAQLR""REIGAQLR" or "EIGAQLR" wherein some positions may be absent
  MOD_RES 14: note = Any amino acid
  MOD_RES 15: note = Met or norleucine
  MOD_RES 18: note = Any amino acid
  REGION 19..24: note = MISC_FEATURE - This region may encompass "LNAQYE" or "LNAQY"wherein some positions may be absent
  SITE 24: note = MISC_FEATURE - May or may not be present
  MOD_RES 25: note = Any cell permeability enhancing amino acid (e.g., amino acidsthat change or shift the distribution of charge or hydrophobiccharacter) or a stability enhancing amino acid (e.g., non-native, D, or alpha methyl amino acid point mutations)
  REGION 1..25: note = See specification as filed for detailed description ofsubstitutions and preferred embodiments
XEQWAREIGAQLRXXADXLNAQYEX

SEQ ID NO: 180 - protein, 26 aa, synthetic construct
  REGION 1..26: note = Description of Artificial Sequence: Syntheticpeptide
  MOD_RES 1: note = beta-Ala
  MOD_RES 14: note = Any non-natural amino acid
  MOD_RES 18: note = Any non-natural amino acid
AAELEVECATQLRXFGDXLNFRQKLL

SEQ ID NO: 181 - protein, 26 aa, synthetic construct
  REGION 1..26: note = Description of Artificial Sequence: Syntheticpeptide
  MOD_RES 1: note = beta-Ala
  MOD_RES 14: note = Any non-natural amino acid
  MOD_RES 18: note = Any non-natural amino acid
AAELEVECATQLRXFGDXLNFRQKLL

SEQ ID NO: 182 - protein, 26 aa, synthetic construct
  REGION 1..26: note = Description of Artificial Sequence: Syntheticpeptide
  MOD_RES 1: note = beta-Ala
  MOD_RES 14: note = Any non-natural amino acid
  MOD_RES 18: note = Any non-natural amino acid
AAELEVESATQLRXFGDXLNFRQKLL

SEQ ID NO: 183 - protein, 26 aa, synthetic construct
  REGION 1..26: note = Description of Artificial Sequence: Syntheticpeptide
  MOD_RES 1: note = beta-Ala
  MOD_RES 14: note = Any non-natural amino acid
  MOD_RES 18: note = Any non-natural amino acid
AAELEVESATQLRXFGDXLNFRQKLL

SEQ ID NO: 184 - protein, 23 aa, synthetic construct
  REGION 1..23: note = Description of Artificial Sequence: Syntheticpeptide
  MOD_RES 10: note = Any non-natural amino acid
  MOD_RES 14: note = Any non-natural amino acid
EVESATQLRXFGDXLNFRQKLLK

SEQ ID NO: 185 - protein, 23 aa, synthetic construct
  REGION 1..23: note = Description of Artificial Sequence: Syntheticpeptide
  MOD_RES 10: note = Any non-natural amino acid
  MOD_RES 14: note = Any non-natural amino acid
EVESATQLRXFGDXLNFRQKLLK

SEQ ID NO: 186 - protein, 22 aa, synthetic construct
  REGION 1..22: note = Description of Artificial Sequence: Syntheticpeptide
  MOD_RES 10: note = Any non-natural amino acid
  MOD_RES 14: note = Any non-natural amino acid
EVESATQLRXFGDXLNFRQKLL

SEQ ID NO: 187 - protein, 23 aa, synthetic construct
  REGION 1..23: note = Description of Artificial Sequence: Syntheticpeptide
  MOD_RES 10: note = Any non-natural amino acid
  MOD_RES 14: note = Any non-natural amino acid
EVESATQLRXFGDXLNFRQKLLK

SEQ ID NO: 188 - protein, 23 aa, synthetic construct
  REGION 1..23: note = Description of Artificial Sequence: Syntheticpeptide
  MOD_RES 10: note = Any non-natural amino acid
  MOD_RES 14: note = Any non-natural amino acid
EVESATQLRXFGDXLNFRQKLLK

SEQ ID NO: 189 - protein, 23 aa, synthetic construct
  REGION 1..23: note = Description of Artificial Sequence: Syntheticpeptide
  MOD_RES 10: note = Any non-natural amino acid
  MOD_RES 14: note = Any non-natural amino acid
EVESATQLRXFGDXLNFRQKLLK

SEQ ID NO: 190 - protein, 23 aa, synthetic construct
  REGION 1..23: note = Description of Artificial Sequence: Syntheticpeptide
  MOD_RES 10: note = Any non-natural amino acid
  MOD_RES 14: note = Any non-natural amino acid
EVESATQLRXFGDXLNFRQKLLK

SEQ ID NO: 191 - protein, 23 aa, synthetic construct
  REGION 1..23: note = Description of Artificial Sequence: Syntheticpeptide
  MOD_RES 10: note = Any non-natural amino acid
  MOD_RES 14: note = Any non-natural amino acid
EVESATQLRXFGDXLNFRQKLLK

SEQ ID NO: 192 - protein, 23 aa, synthetic construct
  REGION 1..23: note = Description of Artificial Sequence: Syntheticpeptide
  MOD_RES 10: note = Any non-natural amino acid
  MOD_RES 14: note = Any non-natural amino acid
EVESATQLRXFGDXLNFRQKLLK

SEQ ID NO: 193 - protein, 22 aa, synthetic construct
  REGION 1..22: note = Description of Artificial Sequence: Syntheticpeptide
  MOD_RES 10: note = Any non-natural amino acid
  MOD_RES 14: note = Any non-natural amino acid
EVESATQLRXFGDXLNFRQKLL

SEQ ID NO: 194 - protein, 23 aa, synthetic construct
  REGION 1..23: note = Description of Artificial Sequence: Syntheticpeptide
  MOD_RES 10: note = Any non-natural amino acid
  MOD_RES 14: note = Any non-natural amino acid
EVESATQLRXFGDXLNFRQKLLK

SEQ ID NO: 195 - protein, 19 aa, synthetic construct
  REGION 1..19: note = Description of Artificial Sequence: Syntheticpeptide
  MOD_RES 7: note = Any non-natural amino acid
  MOD_RES 11: note = Any non-natural amino acid
IAQELRXIGDXFNAYYARK

SEQ ID NO: 196 - protein, 19 aa, synthetic construct
  REGION 1..19: note = Description of Artificial Sequence: Syntheticpeptide
  MOD_RES 7: note = Any non-natural amino acid
  MOD_RES 11: note = Any non-natural amino acid
IAQELRXIGDXFNAYYARK

SEQ ID NO: 197 - protein, 19 aa, synthetic construct
  REGION 1..19: note = Description of Artificial Sequence: Syntheticpeptide
  MOD_RES 7: note = Any non-natural amino acid
  MOD_RES 11: note = Any non-natural amino acid
IAQELRXIGDXFNAYYARR

SEQ ID NO: 198 - protein, 20 aa, synthetic construct
  REGION 1..20: note = Description of Artificial Sequence: Syntheticpeptide
  MOD_RES 7: note = Any non-natural amino acid
  MOD_RES 11: note = Any non-natural amino acid
IAQELRXIGDXFNAYYARRK

SEQ ID NO: 199 - protein, 19 aa, synthetic construct
  REGION 1..19: note = Description of Artificial Sequence: Syntheticpeptide
  MOD_RES 7: note = Any non-natural amino acid
  MOD_RES 11: note = Any non-natural amino acid
IAQELRXIGDXFNAYYARK

SEQ ID NO: 200 - protein, 19 aa, synthetic construct
  REGION 1..19: note = Description of Artificial Sequence: Syntheticpeptide
  MOD_RES 7: note = Any non-natural amino acid
  MOD_RES 11: note = Any non-natural amino acid
IAQELRXIGDXFNAYYARK

SEQ ID NO: 201 - protein, 19 aa, synthetic construct
  REGION 1..19: note = Description of Artificial Sequence: Syntheticpeptide
  MOD_RES 7: note = Any non-natural amino acid
  MOD_RES 11: note = Any non-natural amino acid
IAQELRXIGDXFNAYYARK

SEQ ID NO: 202 - protein, 19 aa, synthetic construct
  REGION 1..19: note = Description of Artificial Sequence: Syntheticpeptide
  MOD_RES 7: note = Any non-natural amino acid
  MOD_RES 11: note = Any non-natural amino acid
IAQELRXIGDXFNAYYARK

SEQ ID NO: 203 - protein, 19 aa, synthetic construct
  REGION 1..19: note = Description of Artificial Sequence: Syntheticpeptide
  MOD_RES 7: note = Any non-natural amino acid
  MOD_RES 11: note = Any non-natural amino acid
IAQELRXIGDXFANYYARK

SEQ ID NO: 204 - protein, 19 aa, synthetic construct
  REGION 1..19: note = Description of Artificial Sequence: Syntheticpeptide
  MOD_RES 7: note = Any non-natural amino acid
  MOD_RES 11: note = Any non-natural amino acid
IAQELRXIGDXFNAYYARR

SEQ ID NO: 205 - protein, 20 aa, synthetic construct
  REGION 1..20: note = Description of Artificial Sequence: Syntheticpeptide
  MOD_RES 7: note = Any non-natural amino acid
  MOD_RES 11: note = Any non-natural amino acid
IAQELRXIGDXFNAYYARRK

SEQ ID NO: 206 - protein, 22 aa, synthetic construct
  REGION 1..22: note = Description of Artificial Sequence: Syntheticpeptide
  MOD_RES 1: note = beta-Ala
  MOD_RES 10: note = Any non-natural amino acid
  MOD_RES 14: note = Any non-natural amino acid
AIWIAQELRXIGDXFNAYYARR

SEQ ID NO: 207 - protein, 19 aa, synthetic construct
  REGION 1..19: note = Description of Artificial Sequence: Syntheticpeptide
  MOD_RES 7: note = Any non-natural amino acid
  MOD_RES 11: note = Any non-natural amino acid
IAQELRXIGDXFNAYYARR

SEQ ID NO: 208 - protein, 21 aa, synthetic construct
  REGION 1..21: note = Description of Artificial Sequence: Syntheticpeptide
  MOD_RES 9: note = Any non-natural amino acid
  MOD_RES 13: note = Any non-natural amino acid
IWIAQELRXIGDXFNAYYARR

SEQ ID NO: 209 - protein, 25 aa, synthetic construct
  REGION 1..25: note = Description of Artificial Sequence: Syntheticpeptide
AELEVECATQLRRFGDKLNFRQKLL

SEQ ID NO: 210 - protein, 9 aa, synthetic construct
  REGION 1..9: note = Description of Artificial Sequence: Synthetic9xHis tag
HHHHHHHHH